European Patent Application EP 4 733 317 A2, published April 29, 2026. Title: NEUTRALIZING ANTI-INFLUENZA B ANTIBODIES AND USES THEREOF. Applicant: MEDIMMUNE, LLC. Application EP, filed July 14, 2015. The sequence listing filed with the application follows.

SEQUENCE LISTING (154 sequences)

SEQ ID NO: 1 - DNA, 391 bp, synthetic construct
  misc_feature 1..391: note = Description of Artificial Sequence: Synthetic polynucleotide
  source 1..391: mol_type = other DNA
gaagtgcagctggtggagtctgggggacacttggtgcagcctggcaggtccctgagactctcctgtgcagcctctggattcacctttgaggattatgccatgaattgggtccggcaagctccagggaagggcctggagtgggtctcagtcattagttgggacagtggtaggataggctatgcggactctgtgaagggccgattcaccatctccagagacaacgccaagaactcctcgtatctgcaaatgaacagtctgagacctgaggacactgccttgtattattgtgtaagagatatgttggcttattattctgacaatagtggcaaaaaatacaacgtctacggtatggacgtctggggccaagggaccacggtcaccgtctcctcag

SEQ ID NO: 2 - protein, 130 aa, synthetic construct
  REGION 1..130: note = Description of Artificial Sequence: Synthetic polypeptide
EVQLVESGGHLVQPGRSLRLSCAASGFTFEDYAMNWVRQAPGKGLEWVSVISWDSGRIGYADSVKGRFTISRDNAKNSSYLQMNSLRPEDTALYYCVRDMLAYYSDNSGKKYNVYGMDVWGQGTTVTVSS

SEQ ID NO: 3 - protein, 5 aa, synthetic construct
  REGION 1..5: note = Description of Artificial Sequence: Synthetic peptide
DYAMN

SEQ ID NO: 4 - protein, 17 aa, synthetic construct
  REGION 1..17: note = Description of Artificial Sequence: Synthetic peptide
VISWDSGRIGYADSVKG

SEQ ID NO: 5 - protein, 21 aa, synthetic construct
  REGION 1..21: note = Description of Artificial Sequence: Synthetic peptide
DMLAYYSDNSGKKYNVYGMDV

SEQ ID NO: 6 - DNA, 322 bp, synthetic construct
  misc_feature 1..322: note = Description of Artificial Sequence: Synthetic polynucleotide
  source 1..322: mol_type = other DNA
gaaattgtgttgacacagtctccagccaccctgtctttgtctccaggggaaagagccaccctctcctgcagggccagtcagagtgtttccaccttcttagcctggtaccaacagaaacctggccaggctcccaggctcctcatgtatgatgcatccaacagggccactggcatcccagccaggttcagtggcagtgggtctgggacagacttcactctcaccatcagcagcctagaacctgaagattttgcaatttactactgtcagcagcgtagccactggcctcctatcttcggccaagggacacgactggagattaaac

SEQ ID NO: 7 - protein, 107 aa, synthetic construct
  REGION 1..107: note = Description of Artificial Sequence: Synthetic polypeptide
EIVLTQSPATLSLSPGERATLSCRASQSVSTFLAWYQQKPGQAPRLLMYDASNRATGIPARFSGSGSGTDFTLTISSLEPEDFAIYYCQQRSHWPPIFGQGTRLEIK

SEQ ID NO: 8 - protein, 10 aa, synthetic construct
  REGION 1..10: note = Description of Artificial Sequence: Synthetic peptide
ASQSVSTFLA

SEQ ID NO: 9 - protein, 7 aa, synthetic construct
  REGION 1..7: note = Description of Artificial Sequence: Synthetic peptide
DASNRAT

SEQ ID NO: 10 - protein, 9 aa, synthetic construct
  REGION 1..9: note = Description of Artificial Sequence: Synthetic peptide
QQRSHWPPI

SEQ ID NO: 11 - DNA, 391 bp, synthetic construct
  misc_feature 1..391: note = Description of Artificial Sequence: Synthetic polynucleotide
  source 1..391: mol_type = other DNA
gaagtgcagctggtggagtctgggggaggcttggtgcaacctggcaggtccctgagactctcctgtgcagtttctggattcatctttgaagattatgccataaactgggtccggcaagctccagggaagggcctggagtgggtctcaattattagttgggacagtggtaggataggctacgcggactctgtgaggggccgattcaccatctccagagacaacgccaagaactcctcgtttctgcaaatgaacagtctgagacccgaagacacggccgtgtattattgtgtaaaagatatgttggcgtattattatgatggtagcggcatcaggtacaacctctacggtatggacgtctggggccaagggaccacggtcaccgtctcctcag

SEQ ID NO: 12 - protein, 130 aa, synthetic construct
  REGION 1..130: note = Description of Artificial Sequence: Synthetic polypeptide
EVQLVESGGGLVQPGRSLRLSCAVSGFIFEDYAINWVRQAPGKGLEWVSIISWDSGRIGYADSVRGRFTISRDNAKNSSFLQMNSLRPEDTAVYYCVKDMLAYYYDGSGIRYNLYGMDVWGQGTTVTVSS

SEQ ID NO: 13 - protein, 5 aa, synthetic construct
  REGION 1..5: note = Description of Artificial Sequence: Synthetic peptide
DYAIN

SEQ ID NO: 14 - protein, 17 aa, synthetic construct
  REGION 1..17: note = Description of Artificial Sequence: Synthetic peptide
IISWDSGRIGYADSVRG

SEQ ID NO: 15 - protein, 21 aa, synthetic construct
  REGION 1..21: note = Description of Artificial Sequence: Synthetic peptide
DMLAYYYDGSGIRYNLYGMDV

SEQ ID NO: 16 - DNA, 322 bp, synthetic construct
  misc_feature 1..322: note = Description of Artificial Sequence: Synthetic polynucleotide
  source 1..322: mol_type = other DNA
gaaattgtgttgacacagtctccagccactctgtctttgtctccaggggaaagagccaccctctcctgcagggccagtcggagtattaccaccttcttagcctggtaccaacaaaaacctggccaggctcccaggctcctcatctacgatgcatccaacagggccactggcgtcccagccaggttcagtggcagtgggtctgggacagacttcactctcaccatcaacagcctagagcctgacgattttgcaatttattactgtcagcagcgtgaccactggcctccgatcttcggccaagggacacgactggagattaaac

SEQ ID NO: 17 - protein, 107 aa, synthetic construct
  REGION 1..107: note = Description of Artificial Sequence: Synthetic polypeptide
EIVLTQSPATLSLSPGERATLSCRASRSITTFLAWYQQKPGQAPRLLIYDASNRATGVPARFSGSGSGTDFTLTINSLEPDDFAIYYCQQRDHWPPIFGQGTRLEIK

SEQ ID NO: 18 - protein, 11 aa, synthetic construct
  REGION 1..11: note = Description of Artificial Sequence: Synthetic peptide
RASRSITTFLA

SEQ ID NO: 19 - protein, 7 aa, synthetic construct
  REGION 1..7: note = Description of Artificial Sequence: Synthetic peptide
DASNRAT

SEQ ID NO: 20 - protein, 9 aa, synthetic construct
  REGION 1..9: note = Description of Artificial Sequence: Synthetic peptide
QQRDHWPPI

SEQ ID NO: 21 - DNA, 403 bp, synthetic construct
  misc_feature 1..403: note = Description of Artificial Sequence: Synthetic polynucleotide
  source 1..403: mol_type = other DNA
gaggtgcagctggtggtgtctgggggaggcttggtaaagcctggggggtcccttagactctcctgtgcagcctctggactcagtttccttaacgcctggatgagctgggtccgccaggctccagggaaggggctggagtgggttggccgtattaaaagtaatactgatggtgggacaacagactacgccgcacccgtgaaaggcagattcagcatctcaagagacgattcaaagaacatgctgtttctgcatatgagcagcctgagaaccgaggacacagccgtctattactgcgccacagatggaccttactctgacgattttagaagtggttatgccgcacgctaccgttatttcggaatggacgtctggggccaagggaccacggtcaccgtctcctcag

SEQ ID NO: 22 - protein, 134 aa, synthetic construct
  REGION 1..134: note = Description of Artificial Sequence: Synthetic polypeptide
EVQLVVSGGGLVKPGGSLRLSCAASGLSFLNAWMSWVRQAPGKGLEWVGRIKSNTDGGTTDYAAPVKGRFSISRDDSKNMLFLHMSSLRTEDTAVYYCATDGPYSDDFRSGYAARYRYFGMDVWGQGTTVTVSS

SEQ ID NO: 23 - protein, 5 aa, synthetic construct
  REGION 1..5: note = Description of Artificial Sequence: Synthetic peptide
NAWMS

SEQ ID NO: 24 - protein, 19 aa, synthetic construct
  REGION 1..19: note = Description of Artificial Sequence: Synthetic peptide
RIKSNTDGGTTDYAAPVKG

SEQ ID NO: 25 - protein, 23 aa, synthetic construct
  REGION 1..23: note = Description of Artificial Sequence: Synthetic peptide
DGPYSDDFRSGYAARYRYFGMDV

SEQ ID NO: 26 - DNA, 322 bp, synthetic construct
  misc_feature 1..322: note = Description of Artificial Sequence: Synthetic polynucleotide
  source 1..322: mol_type = other DNA
gacatccagatgacccagtctccatcttccgtgtctgcatctgtgggagacagagtcaccatcacttgtcgggcgagtcaggatattagcacctggttagcctggtatcagcagaaaccagggaaagcccctaagctcctgatctatgctgcatccagtttgcaaagtggggtcccatcaagattcagcggcagtggatctgggacagatttcactctcaccatcagcagcctgcagcctgaagattttgcaacttacttttgtcagcaggctaacagtttccctccgacttttggccaggggaccaagctggagatcaaac

SEQ ID NO: 27 - protein, 107 aa, synthetic construct
  REGION 1..107: note = Description of Artificial Sequence: Synthetic polypeptide
DIQMTQSPSSVSASVGDRVTITCRASQDISTWLAWYQQKPGKAPKLLIYAASSLQSGVPSRFSGSGSGTDFTLTISSLQPEDFATYFCQQANSFPPTFGQGTKLEIK

SEQ ID NO: 28 - protein, 11 aa, synthetic construct
  REGION 1..11: note = Description of Artificial Sequence: Synthetic peptide
RASQDISTWLA

SEQ ID NO: 29 - protein, 7 aa, synthetic construct
  REGION 1..7: note = Description of Artificial Sequence: Synthetic peptide
AASSLQS

SEQ ID NO: 30 - protein, 9 aa, synthetic construct
  REGION 1..9: note = Description of Artificial Sequence: Synthetic peptide
QQANSFPPT

SEQ ID NO: 31 - DNA, 402 bp, synthetic construct
  misc_feature 1..402: note = Description of Artificial Sequence: Synthetic polynucleotide
  source 1..402: mol_type = other DNA
gaggtgcagctggtggagtctgggggaggcttggtaaagcctggggggtcccttagactctcctgtgcagcctctggactctctttccttaacgcctggatgagctgggtccgccaggctccagggaagggcctggagtgggttggccgtattaaaagtaatactgatggtgggacaacagactacgccgcacccgtgaaaggcagattcaccatctcaagagacgattcaaagaacacgctgtatctgcaaatgagcagcctgaaaaccgaggacacagccgtctattactgcaccacagatggaccttactctgacgattttagaagtggttatgccgcacgctaccgttatttcggaatggacgtctggggccaagggaccacggtcaccgtctcctca

SEQ ID NO: 32 - protein, 134 aa, synthetic construct
  REGION 1..134: note = Description of Artificial Sequence: Synthetic polypeptide
EVQLVESGGGLVKPGGSLRLSCAASGLSFLNAWMSWVRQAPGKGLEWVGRIKSNTDGGTTDYAAPVKGRFTISRDDSKNTLYLQMSSLKTEDTAVYYCTTDGPYSDDFRSGYAARYRYFGMDVWGQGTTVTVSS

SEQ ID NO: 33 - protein, 5 aa, synthetic construct
  REGION 1..5: note = Description of Artificial Sequence: Synthetic peptide
NAWMS

SEQ ID NO: 34 - protein, 19 aa, synthetic construct
  REGION 1..19: note = Description of Artificial Sequence: Synthetic peptide
RIKSNTDGGTTDYAAPVKG

SEQ ID NO: 35 - protein, 23 aa, synthetic construct
  REGION 1..23: note = Description of Artificial Sequence: Synthetic peptide
DGPYSDDFRSGYAARYRYFGMDV

SEQ ID NO: 36 - DNA, 322 bp, synthetic construct
  misc_feature 1..322: note = Description of Artificial Sequence: Synthetic polynucleotide
  source 1..322: mol_type = other DNA
gacatccagatgacccagtctccatcttccgtgtctgcatctgtgggagacagagtcaccatcacttgtcgggcgagtcaggatattagcacctggttagcctggtatcagcagaaaccagggaaagcccctaagctcctgatctatgctgcatccagtttgcaaagtggggtcccatcaagattcagcggcagtggatctgggacagatttcactctcaccatcagcagcctgcagcctgaagattttgcaacttactattgtcagcaggctaacagtttccctccgacttttggccaggggaccaagctggagatcaaac

SEQ ID NO: 37 - protein, 107 aa, synthetic construct
  REGION 1..107: note = Description of Artificial Sequence: Synthetic polypeptide
DIQMTQSPSSVSASVGDRVTITCRASQDISTWLAWYQQKPGKAPKLLIYAASSLQSGVPSRFSGSGSGTDFTLTISSLQPEDFATYYCQQANSFPPTFGQGTKLEIK

SEQ ID NO: 38 - protein, 11 aa, synthetic construct
  REGION 1..11: note = Description of Artificial Sequence: Synthetic peptide
RASQDISTWLA

SEQ ID NO: 39 - protein, 7 aa, synthetic construct
  REGION 1..7: note = Description of Artificial Sequence: Synthetic peptide
AASSLQS

SEQ ID NO: 40 - protein, 9 aa, synthetic construct
  REGION 1..9: note = Description of Artificial Sequence: Synthetic peptide
QQANSFPPT

SEQ ID NO: 41 - DNA, 402 bp, synthetic construct
  misc_feature 1..402: note = Description of Artificial Sequence: Synthetic polynucleotide
  source 1..402: mol_type = other DNA
gaggtgcagctggtggagtctgggggaggcttggtaaagcctggggggtcccttagactctcctgtgcagcctctggattctctttccttaacgcctggatgagctgggtccgccaggctccagggaagggcctggagtgggttggccgtattaaaagtaatactgatggtgggacaacagactacgccgcacccgtgaaaggcagattcaccatctcaagagacgattcaaagaacacgctgtatctgcaaatgagcagcctgaaaaccgaggacacagccgtctattactgcaccacagatggaccttactctgacgattttagaagtggttatgccgcacgctaccgttatttcggaatggacgtctggggccaagggaccacggtcaccgtctcctca

SEQ ID NO: 42 - protein, 134 aa, synthetic construct
  REGION 1..134: note = Description of Artificial Sequence: Synthetic polypeptide
EVQLVESGGGLVKPGGSLRLSCAASGFSFLNAWMSWVRQAPGKGLEWVGRIKSNTDGGTTDYAAPVKGRFTISRDDSKNTLYLQMSSLKTEDTAVYYCTTDGPYSDDFRSGYAARYRYFGMDVWGQGTTVTVSS

SEQ ID NO: 43 - protein, 5 aa, synthetic construct
  REGION 1..5: note = Description of Artificial Sequence: Synthetic peptide
NAWMS

SEQ ID NO: 44 - protein, 19 aa, synthetic construct
  REGION 1..19: note = Description of Artificial Sequence: Synthetic peptide
RIKSNTDGGTTDYAAPVKG

SEQ ID NO: 45 - protein, 23 aa, synthetic construct
  REGION 1..23: note = Description of Artificial Sequence: Synthetic peptide
DGPYSDDFRSGYAARYRYFGMDV

SEQ ID NO: 46 - DNA, 322 bp, synthetic construct; identical to SEQ ID NO: 36
  misc_feature 1..322: note = Description of Artificial Sequence: Synthetic polynucleotide
  source 1..322: mol_type = other DNA

SEQ ID NO: 47 - protein, 107 aa, synthetic construct; identical to SEQ ID NO: 37
  REGION 1..107: note = Description of Artificial Sequence: Synthetic polypeptide

SEQ ID NO: 48 - protein, 11 aa, synthetic construct
  REGION 1..11: note = Description of Artificial Sequence: Synthetic peptide
RASQDISTWLA

SEQ ID NO: 49 - protein, 7 aa, synthetic construct
  REGION 1..7: note = Description of Artificial Sequence: Synthetic peptide
AASSLQS

SEQ ID NO: 50 - protein, 9 aa, synthetic construct
  REGION 1..9: note = Description of Artificial Sequence: Synthetic peptide
QQANSFPPT

SEQ ID NO: 51 - DNA, 402 bp, synthetic construct
  misc_feature 1..402: note = Description of Artificial Sequence: Synthetic polynucleotide
  source 1..402: mol_type = other DNA
gaggtgcagctggtggagtctgggggaggcttggtaaagcctggggggtcccttagactctcctgtgcagcctctggactcactttccttaacgcctggatgagctgggtccgccaggctccagggaagggcctggagtgggttggccgtattaaaagtaatactgatggtgggacaacagactacgccgcacccgtgaaaggcagattcaccatctcaagagacgattcaaagaacacgctgtatctgcaaatgagcagcctgaaaaccgaggacacagccgtctattactgcaccacagatggaccttactctgacgattttagaagtggttatgccgcacgctaccgttatttcggaatggacgtctggggccaagggaccacggtcaccgtctcctca

SEQ ID NO: 52 - protein, 134 aa, synthetic construct
  REGION 1..134: note = Description of Artificial Sequence: Synthetic polypeptide
EVQLVESGGGLVKPGGSLRLSCAASGLTFLNAWMSWVRQAPGKGLEWVGRIKSNTDGGTTDYAAPVKGRFTISRDDSKNTLYLQMSSLKTEDTAVYYCTTDGPYSDDFRSGYAARYRYFGMDVWGQGTTVTVSS

SEQ ID NO: 53 - protein, 5 aa, synthetic construct
  REGION 1..5: note = Description of Artificial Sequence: Synthetic peptide
NAWMS

SEQ ID NO: 54 - protein, 19 aa, synthetic construct
  REGION 1..19: note = Description of Artificial Sequence: Synthetic peptide
RIKSNTDGGTTDYAAPVKG

SEQ ID NO: 55 - protein, 23 aa, synthetic construct
  REGION 1..23: note = Description of Artificial Sequence: Synthetic peptide
DGPYSDDFRSGYAARYRYFGMDV

SEQ ID NO: 56 - DNA, 322 bp, synthetic construct; identical to SEQ ID NO: 36
  misc_feature 1..322: note = Description of Artificial Sequence: Synthetic polynucleotide
  source 1..322: mol_type = other DNA

SEQ ID NO: 57 - protein, 107 aa, synthetic construct; identical to SEQ ID NO: 37
  REGION 1..107: note = Description of Artificial Sequence: Synthetic polypeptide

SEQ ID NO: 58 - protein, 11 aa, synthetic construct
  REGION 1..11: note = Description of Artificial Sequence: Synthetic peptide
RASQDISTWLA

SEQ ID NO: 59 - protein, 7 aa, synthetic construct
  REGION 1..7: note = Description of Artificial Sequence: Synthetic peptide
AASSLQS

SEQ ID NO: 60 - protein, 9 aa, synthetic construct
  REGION 1..9: note = Description of Artificial Sequence: Synthetic peptide
QQANSFPPT

SEQ ID NO: 61 - DNA, 402 bp, synthetic construct
  misc_feature 1..402: note = Description of Artificial Sequence: Synthetic polynucleotide
  source 1..402: mol_type = other DNA
gaggtgcagctggtggagtctgggggaggcttggtaaagcctggggggtcccttagactctcctgtgcagcctctggattcactttccttaacgcctggatgagctgggtccgccaggctccagggaagggcctggagtgggttggccgtattaaaagtaatactgatggtgggacaacagactacgccgcacccgtgaaaggcagattcaccatctcaagagacgattcaaagaacacgctgtatctgcaaatgagcagcctgaaaaccgaggacacagccgtctattactgcaccacagatggaccttactctgacgattttagaagtggttatgccgcacgctaccgttatttcggaatggacgtctggggccaagggaccacggtcaccgtctcctca

SEQ ID NO: 62 - protein, 134 aa, synthetic construct
  REGION 1..134: note = Description of Artificial Sequence: Synthetic polypeptide
EVQLVESGGGLVKPGGSLRLSCAASGFTFLNAWMSWVRQAPGKGLEWVGRIKSNTDGGTTDYAAPVKGRFTISRDDSKNTLYLQMSSLKTEDTAVYYCTTDGPYSDDFRSGYAARYRYFGMDVWGQGTTVTVSS

SEQ ID NO: 63 - protein, 5 aa, synthetic construct
  REGION 1..5: note = Description of Artificial Sequence: Synthetic peptide
NAWMS

SEQ ID NO: 64 - protein, 19 aa, synthetic construct
  REGION 1..19: note = Description of Artificial Sequence: Synthetic peptide
RIKSNTDGGTTDYAAPVKG

SEQ ID NO: 65 - protein, 23 aa, synthetic construct
  REGION 1..23: note = Description of Artificial Sequence: Synthetic peptide
DGPYSDDFRSGYAARYRYFGMDV

SEQ ID NO: 66 - DNA, 322 bp, synthetic construct; identical to SEQ ID NO: 36
  misc_feature 1..322: note = Description of Artificial Sequence: Synthetic polynucleotide
  source 1..322: mol_type = other DNA

SEQ ID NO: 67 - protein, 107 aa, synthetic construct; identical to SEQ ID NO: 37
  REGION 1..107: note = Description of Artificial Sequence: Synthetic polypeptide

SEQ ID NO: 68 - protein, 11 aa, synthetic construct
  REGION 1..11: note = Description of Artificial Sequence: Synthetic peptide
RASQDISTWLA

SEQ ID NO: 69 - protein, 7 aa, synthetic construct
  REGION 1..7: note = Description of Artificial Sequence: Synthetic peptide
AASSLQS

SEQ ID NO: 70 - protein, 9 aa, synthetic construct
  REGION 1..9: note = Description of Artificial Sequence: Synthetic peptide
QQANSFPPT

SEQ ID NO: 71 - protein, 134 aa, synthetic construct
  REGION 1..134: note = Description of Artificial Sequence: Synthetic polypeptide
  MOD_RES 6: note = Val or Glu
  MOD_RES 27: note = Leu or Phe
  MOD_RES 28: note = Thr or Ser
  MOD_RES 30: note = Ser or Leu
  MOD_RES 71: note = Thr or Ser
  MOD_RES 80: note = Thr or Met
  MOD_RES 82: note = Tyr or Phe
  MOD_RES 84: note = Gln or His
  MOD_RES 86: note = Asn or Ser
  MOD_RES 89: note = Lys or Arg
  MOD_RES 99: note = Thr or Ala
EVQLVXSGGGLVKPGGSLRLSCAASGXXFXNAWMSWVRQAPGKGLEWVGRIKSNTDGGTTDYAAPVKGRFXISRDDSKNXLXLXMXSLXTEDTAVYYCXTDGPYSDDFRSGYAARYRYFGMDVWGQGTTVTVSS

SEQ ID NO: 72 - protein, 107 aa, synthetic construct
  REGION 1..107: note = Description of Artificial Sequence: Synthetic polypeptide
  MOD_RES 87: note = Phe or Tyr
DIQMTQSPSSVSASVGDRVTITCRASQDISTWLAWYQQKPGKAPKLLIYAASSLQSGVPSRFSGSGSGTDFTLTISSLQPEDFATYXCQQANSFPPTFGQGTKLEIK

SEQ ID NO: 73 - DNA, 402 bp, synthetic construct
  misc_feature 1..402: note = Description of Artificial Sequence: Synthetic polynucleotide
  source 1..402: mol_type = other DNA
gaggtgcagctggtggagtctgggggaggcttggtaaagcctggggggtcccttagactctcctgtgcagcctctggattctctttcagtaacgcctggatgagctgggtccgccaggctccagggaagggcctggagtgggttggccgtattaaaagtaatactgatggtgggacaacagactacgccgcacccgtgaaaggcagattcaccatctcaagagacgattcaaagaacacgctgtatctgcaaatgagcagcctgaaaaccgaggacacagccgtctattactgcaccacagatggaccttactctgacgattttagaagtggttatgccgcacgctaccgttatttcggaatggacgtctggggccaagggaccacggtcaccgtctcctca

SEQ ID NO: 74 - protein, 134 aa, synthetic construct
  REGION 1..134: note = Description of Artificial Sequence: Synthetic polypeptide
EVQLVESGGGLVKPGGSLRLSCAASGFSFSNAWMSWVRQAPGKGLEWVGRIKSNTDGGTTDYAAPVKGRFTISRDDSKNTLYLQMSSLKTEDTAVYYCTTDGPYSDDFRSGYAARYRYFGMDVWGQGTTVTVSS

SEQ ID NO: 75 - protein, 11 aa, synthetic construct
  REGION 1..11: note = Description of Artificial Sequence: Synthetic peptide
RASQDISTWLA

SEQ ID NO: 76 - protein, 19 aa, synthetic construct
  REGION 1..19: note = Description of Artificial Sequence: Synthetic peptide
RIKSNTDGGTTDYAAPVKG

SEQ ID NO: 77 - protein, 23 aa, synthetic construct
  REGION 1..23: note = Description of Artificial Sequence: Synthetic peptide
DGPYSDDFRSGYAARYRYFGMDV

SEQ ID NO: 78 - protein, 8 aa, synthetic construct
  REGION 1..8: note = Description of Artificial Sequence: Synthetic peptide
GFSFSNAW

SEQ ID NO: 79 - protein, 10 aa, synthetic construct
  REGION 1..10: note = Description of Artificial Sequence: Synthetic peptide
IKSNTDGGTT

SEQ ID NO: 80 - protein, 25 aa, synthetic construct
  REGION 1..25: note = Description of Artificial Sequence: Synthetic peptide
TTDGPYSDDFRSGYAARYRYFGMDV

SEQ ID NO: 81 - DNA, 322 bp, synthetic construct; identical to SEQ ID NO: 36
  misc_feature 1..322: note = Description of Artificial Sequence: Synthetic polynucleotide
  source 1..322: mol_type = other DNA

SEQ ID NO: 82 - protein, 107 aa, synthetic construct; identical to SEQ ID NO: 37
  REGION 1..107: note = Description of Artificial Sequence: Synthetic polypeptide

SEQ ID NO: 83 - protein, 11 aa, synthetic construct
  REGION 1..11: note = Description of Artificial Sequence: Synthetic peptide
RASQDISTWLA

SEQ ID NO: 84 - protein, 7 aa, synthetic construct
  REGION 1..7: note = Description of Artificial Sequence: Synthetic peptide
AASSLQS

SEQ ID NO: 85 - protein, 9 aa, synthetic construct
  REGION 1..9: note = Description of Artificial Sequence: Synthetic peptide
QQANSFPPT

SEQ ID NO: 86 - protein, 6 aa, synthetic construct
  REGION 1..6: note = Description of Artificial Sequence: Synthetic peptide
QDISTW

SEQ ID NO: 87 - skipped

SEQ ID NO: 88 - protein, 9 aa, synthetic construct
  REGION 1..9: note = Description of Artificial Sequence: Synthetic peptide
QQANSFPPT

SEQ ID NO: 89 - DNA, 402 bp, synthetic construct
  misc_feature 1..402: note = Description of Artificial Sequence: Synthetic polynucleotide
  source 1..402: mol_type = other DNA
gaggtgcagctggtggagtctgggggaggcttggtaaagcctggggggtcccttagactctcctgtgcagcctctggactcactttcagtaacgcctggatgagctgggtccgccaggctccagggaagggcctggagtgggttggccgtattaaaagtaatactgatggtgggacaacagactacgccgcacccgtgaaaggcagattcaccatctcaagagacgattcaaagaacacgctgtatctgcaaatgagcagcctgaaaaccgaggacacagccgtctattactgcaccacagatggaccttactctgacgattttagaagtggttatgccgcacgctaccgttatttcggaatggacgtctggggccaagggaccacggtcaccgtctcctca

SEQ ID NO: 90 - protein, 134 aa, synthetic construct
  REGION 1..134: note = Description of Artificial Sequence: Synthetic polypeptide
EVQLVESGGGLVKPGGSLRLSCAASGLTFSNAWMSWVRQAPGKGLEWVGRIKSNTDGGTTDYAAPVKGRFTISRDDSKNTLYLQMSSLKTEDTAVYYCTTDGPYSDDFRSGYAARYRYFGMDVWGQGTTVTVSS

SEQ ID NO: 91 - protein, 11 aa, synthetic construct
  REGION 1..11: note = Description of Artificial Sequence: Synthetic peptide
RASQDISTWLA

SEQ ID NO: 92 - protein, 19 aa, synthetic construct
  REGION 1..19: note = Description of Artificial Sequence: Synthetic peptide
RIKSNTDGGTTDYAAPVKG

SEQ ID NO: 93 - protein, 23 aa, synthetic construct
  REGION 1..23: note = Description of Artificial Sequence: Synthetic peptide
DGPYSDDFRSGYAARYRYFGMDV

SEQ ID NO: 94 - protein, 8 aa, synthetic construct
  REGION 1..8: note = Description of Artificial Sequence: Synthetic peptide
GLTFSNAW

SEQ ID NO: 95 - protein, 10 aa, synthetic construct
  REGION 1..10: note = Description of Artificial Sequence: Synthetic peptide
IKSNTDGGTT

SEQ ID NO: 96 - protein, 25 aa, synthetic construct
  REGION 1..25: note = Description of Artificial Sequence: Synthetic peptide
TTDGPYSDDFRSGYAARYRYFGMDV

SEQ ID NO: 97 - DNA, 322 bp, synthetic construct; identical to SEQ ID NO: 36
  misc_feature 1..322: note = Description of Artificial Sequence: Synthetic polynucleotide
  source 1..322: mol_type = other DNA

SEQ ID NO: 98 - protein, 107 aa, synthetic construct; identical to SEQ ID NO: 37
  REGION 1..107: note = Description of Artificial Sequence: Synthetic polypeptide

SEQ ID NO: 99 - protein, 11 aa, synthetic construct
  REGION 1..11: note = Description of Artificial Sequence: Synthetic peptide
RASQDISTWLA

SEQ ID NO: 100 - protein, 7 aa, synthetic construct
  REGION 1..7: note = Description of Artificial Sequence: Synthetic peptide
AASSLQS

SEQ ID NO: 101 - protein, 9 aa, synthetic construct
  REGION 1..9: note = Description of Artificial Sequence: Synthetic peptide
QQANSFPPT

SEQ ID NO: 102 - protein, 6 aa, synthetic construct
  REGION 1..6: note = Description of Artificial Sequence: Synthetic peptide
QDISTW

SEQ ID NO: 103 - skipped

SEQ ID NO: 104 - protein, 9 aa, synthetic construct
  REGION 1..9: note = Description of Artificial Sequence: Synthetic peptide
QQANSFPPT

SEQ ID NO: 105 - DNA, 402 bp, synthetic construct
  misc_feature 1..402: note = Description of Artificial Sequence: Synthetic polynucleotide
  source 1..402: mol_type = other DNA
gaggtgcagctggtggagtctgggggaggcttggtaaagcctggggggtcccttagactctcctgtgcagcctctggattcactttcagtaacgcctggatgagctgggtccgccaggctccagggaagggcctggagtgggttggccgtattaaaagtaatactgatggtgggacaacagactacgccgcacccgtgaaaggcagattcaccatctcaagagacgattcaaagaacacgctgtatctgcaaatgagcagcctgaaaaccgaggacacagccgtctattactgcaccacagatggaccttactctgacgattttagaagtggttatgccgcacgctaccgttatttcggaatggacgtctggggccaagggaccacggtcaccgtctcctca

SEQ ID NO: 106 - protein, 134 aa, synthetic construct
  REGION 1..134: note = Description of Artificial Sequence: Synthetic polypeptide
EVQLVESGGGLVKPGGSLRLSCAASGFTFSNAWMSWVRQAPGKGLEWVGRIKSNTDGGTTDYAAPVKGRFTISRDDSKNTLYLQMSSLKTEDTAVYYCTTDGPYSDDFRSGYAARYRYFGMDVWGQGTTVTVSS

SEQ ID NO: 107 - protein, 11 aa, synthetic construct
  REGION 1..11: note = Description of Artificial Sequence: Synthetic peptide
RASQDISTWLA

SEQ ID NO: 108 - protein, 19 aa, synthetic construct
  REGION 1..19: note = Description of Artificial Sequence: Synthetic peptide
RIKSNTDGGTTDYAAPVKG

SEQ ID NO: 109 - protein, 23 aa, synthetic construct
  REGION 1..23: note = Description of Artificial Sequence: Synthetic peptide
DGPYSDDFRSGYAARYRYFGMDV

SEQ ID NO: 110 - protein, 8 aa, synthetic construct
  REGION 1..8: note = Description of Artificial Sequence: Synthetic peptide
GFTFSNAW

SEQ ID NO: 111 - protein, 10 aa, synthetic construct
  REGION 1..10: note = Description of Artificial Sequence: Synthetic peptide
IKSNTDGGTT

SEQ ID NO: 112 - protein, 24 aa, synthetic construct
  REGION 1..24: note = Description of Artificial Sequence: Synthetic peptide
TDGPYSDDFRSGYAARYRYFGMDV

SEQ ID NO: 113 - DNA, 322 bp, synthetic construct; identical to SEQ ID NO: 36
  misc_feature 1..322: note = Description of Artificial Sequence: Synthetic polynucleotide
  source 1..322: mol_type = other DNA

SEQ ID NO: 114 - protein, 107 aa, synthetic construct; identical to SEQ ID NO: 37
  REGION 1..107: note = Description of Artificial Sequence: Synthetic polypeptide

SEQ ID NO: 115 - protein, 11 aa, synthetic construct
  REGION 1..11: note = Description of Artificial Sequence: Synthetic peptide
RASQDISTWLA

SEQ ID NO: 116 - protein, 7 aa, synthetic construct
  REGION 1..7: note = Description of Artificial Sequence: Synthetic peptide
AASSLQS

SEQ ID NO: 117 - protein, 9 aa, synthetic construct
  REGION 1..9: note = Description of Artificial Sequence: Synthetic peptide
QQANSFPPT

SEQ ID NO: 118 - protein, 6 aa, synthetic construct
  REGION 1..6: note = Description of Artificial Sequence: Synthetic peptide
QDISTW

SEQ ID NO: 119 - skipped

SEQ ID NO: 120 - protein, 9 aa, synthetic construct
  REGION 1..9: note = Description of Artificial Sequence: Synthetic peptide
QQANSFPPT

SEQ ID NO: 121 - protein, 8 aa, synthetic construct
  REGION 1..8: note = Description of Artificial Sequence: Synthetic peptide
GLSFLNAW

SEQ ID NO: 122 - protein, 10 aa, synthetic construct
  REGION 1..10: note = Description of Artificial Sequence: Synthetic peptide
IKSNTDGGTT

SEQ ID NO: 123 - protein, 25 aa, synthetic construct
  REGION 1..25: note = Description of Artificial Sequence: Synthetic peptide
TDGPYSDDFRSGYAARYRYFGMDVW

SEQ ID NO: 124 - protein, 6 aa, synthetic construct
  REGION 1..6: note = Description of Artificial Sequence: Synthetic peptide
QDISTW

SEQ ID NO: 125 - skipped

SEQ ID NO: 126 - protein, 9 aa, synthetic construct
  REGION 1..9: note = Description of Artificial Sequence: Synthetic peptide
QQANSFPPT

SEQ ID NO: 127 - protein, 8 aa, synthetic construct
  REGION 1..8: note = Description of Artificial Sequence: Synthetic peptide
GLSFLNAW

SEQ ID NO: 128 - protein, 10 aa, synthetic construct
  REGION 1..10: note = Description of Artificial Sequence: Synthetic peptide
IKSNTDGGTT

SEQ ID NO: 129 - protein, 25 aa, synthetic construct
  REGION 1..25: note = Description of Artificial Sequence: Synthetic peptide
TTDGPYSDDFRSGYAARYRYFGMDV

SEQ ID NO: 130 - protein, 6 aa, synthetic construct
  REGION 1..6: note = Description of Artificial Sequence: Synthetic peptide
QDISTW

SEQ ID NO: 131 - skipped

SEQ ID NO: 132 - protein, 9 aa, synthetic construct
  REGION 1..9: note = Description of Artificial Sequence: Synthetic peptide
QQANSFPPT

SEQ ID NO: 133 - protein, 8 aa, synthetic construct
  REGION 1..8: note = Description of Artificial Sequence: Synthetic peptide
GFSFLNAW

SEQ ID NO: 134 - protein, 10 aa, synthetic construct
  REGION 1..10: note = Description of Artificial Sequence: Synthetic peptide
IKSNTDGGTT

SEQ ID NO: 135 - protein, 25 aa, synthetic construct
  REGION 1..25: note = Description of Artificial Sequence: Synthetic peptide
TTDGPYSDDFRSGYAARYRYFGMDV

SEQ ID NO: 136 - protein, 6 aa, synthetic construct
  REGION 1..6: note = Description of Artificial Sequence: Synthetic peptide
QDISTW

SEQ ID NO: 137 - skipped

SEQ ID NO: 138 - protein, 9 aa, synthetic construct
  REGION 1..9: note = Description of Artificial Sequence: Synthetic peptide
QQANSFPPT

SEQ ID NO: 139 - protein, 8 aa, synthetic construct
  REGION 1..8: note = Description of Artificial Sequence: Synthetic peptide
GLTFLNAW

SEQ ID NO: 140 - protein, 10 aa, synthetic construct
  REGION 1..10: note = Description of Artificial Sequence: Synthetic peptide
IKSNTDGGTT

SEQ ID NO: 141 - protein, 25 aa, synthetic construct
  REGION 1..25: note = Description of Artificial Sequence: Synthetic peptide
TTDGPYSDDFRSGYAARYRYFGMDV

SEQ ID NO: 142 - protein, 6 aa, synthetic construct
  REGION 1..6: note = Description of Artificial Sequence: Synthetic peptide
QDISTW

SEQ ID NO: 143 - skipped

SEQ ID NO: 144 - protein, 9 aa, synthetic construct
  REGION 1..9: note = Description of Artificial Sequence: Synthetic peptide
QQANSFPPT

SEQ ID NO: 145 - protein, 8 aa, synthetic construct
  REGION 1..8: note = Description of Artificial Sequence: Synthetic peptide
GFTFLNAW

SEQ ID NO: 146 - protein, 10 aa, synthetic construct
  REGION 1..10: note = Description of Artificial Sequence: Synthetic peptide
IKSNTDGGTT

SEQ ID NO: 147 - protein, 25 aa, synthetic construct
  REGION 1..25: note = Description of Artificial Sequence: Synthetic peptide
TTDGPYSDDFRSGYAARYRYFGMDV

SEQ ID NO: 148 - protein, 6 aa, synthetic construct
  REGION 1..6: note = Description of Artificial Sequence: Synthetic peptide
QDISTW

SEQ ID NO: 149 - skipped

SEQ ID NO: 150 - protein, 9 aa, synthetic construct
  REGION 1..9: note = Description of Artificial Sequence: Synthetic peptide
QQANSFPPT

SEQ ID NO: 151 - protein, 347 aa, Influenza B virus
DRICTGITSSNSPHVVKTATQGEVNVTGVIPLTTTPTKSHFANLKGTETRGKLCPKCLNCTDLDVALGRPKCTGNIPSARVSILHEVRPVTSGCFPIMHDRTKIRQLPNLLRGYEHIRLSTHNVINAENAPGGPYKIGTSGSCPNVTNGNGFFATMAWAVPKNDNNKTATNSLTIEVPYICTEGEDQITVWGFHSDNEIQMAKLYGDSKPQKFTSSANGVTTHYVSQIGGFPNQTEDGGLPQSGRIVVDYMVQKSGKTGTITYQRGILLPQKVWCASGRSKVIKGSLPLIGEADCLHEKYGGLNKSKPYYTGEHAKAIGNCPIWVKTPLKLANGTKYRPPAKLLKER

SEQ ID NO: 152 - protein, 346 aa, Influenza B virus
DRICTGITSSNSPHVVKTATQGEVNVTGVIPLTTTPTKSYFANLKGTRTRGKLCPDCLNCTDLDVALGRPMCVGTTPSAKASILHEVKPVTSGCFPIMHDRTKIRQLPNLLRGYENIRLSTQNVIDAEKAPGGPYRLGTSGSCPNATSKSGFFATMAWAVPKDNNKNATNPLTVEVPYICTEGEDQITVWGFHSDDKTQMKNLYGDSNPQKFTSSANGVTTHYVSQIGSFPDQTEDGGLPQSGRIVVDYMMQKPGKTGTIVYQRGVLLPQKVWCASGRSKVIKGSLPLIGEADCLHEKYGGLNKSKPYYTGEHAKAIGNCPIWVKTPLKLANGTKYRPPAKLLKER

SEQ ID NO: 153 - protein, 346 aa, Influenza B virus
DRICTGITSSNSPHVVKTATQGEVNVTGVIPLTTTPTKSYFANLKGTRTRGKLCPDCLNCTDLDVALGRPMCVGTTPSAKASILHEVKPVTSGCFPIMHDRTKIRQLPNLLRGYENIRLSTQNVIDAEKAPGGPYRLGTSESCPNATSKSGFFATMAWAVPKDNNKNATNPLTVEVPYICTEGEDQITVWGFHSDDKTQMKNLYGDSNPQKFTSSANGVTTHYVSQIGSFPDQTEDGGLPQSGRIVVDYMMQKPGKTGTIVYQRGVLLPQKVWCASGRSKVIKGSLPLIGEADCLHEKYGGLNKSKPYYTGEHAKAIGNCPIWVKTPLKLANGTKYRPPAKLLKER

SEQ ID NO: 154 - protein, 346 aa, Influenza B virus
DRICTGITSSNSPHVVKTATQGEVNVTGVIPLTTTPTKSYFANLKGTRTRGKLCPDCLNCTDLDVALGRPMCVGTTPSAKASILHEVRPVTSGCFPIMHDRTKIRQLPNLLRGYENIRLSTQNVIDAENAPGGPYRLGTSRSCPNATSKSGFFATMAWAVPKDNNKNATNPLTVEVPYVCTEGEDQITVWGFHSDNKTQMKNLYGDSNPQKFTSSANGVTTHYVSQIGGFPAQTEDEGLPQSGRIVVDYMVQKPRKTGTIVYQRGVLLPQKVWCASGRSKVIKGSLPLIGEADCLHEKYGGLNKSKPYYTGEHAKAIGNCPIWVKTPLKLANGTKYRPPAKLLKER